European Patent Application EP 4 623 925 A2, published October 1, 2025. Title: PEPTIDE COMPOSITIONS AND METHODS OF USE. Applicant: ONL Therapeutics, Inc. The sequence listing filed with the application follows.

SEQUENCE LISTING (2 sequences)

SEQ ID NO: 1 - protein, 12 aa, synthetic construct
  REGION 1..12: note = artificail peptide; C-terminal amide of Met-12
HHIYLGAVNYIY

SEQ ID NO: 2 - protein, 12 aa, synthetic construct
  REGION 1..12: note = artificial peptide; a small peptide inhibitor, Met-12
HHIYLGAVNYIY